European Patent Application EP 4 498 085 A1, published January 29, 2025. Title: Compositions for preventing or treating cancer including DDX54 inhibitors and immunic cancer agents. Applicant: Korea Advanced Institute of Science and Technology. Application KR. The sequence listing filed with the application follows.

SEQUENCE LISTING (1 sequence)

SEQ ID NO: 1 - DNA, 21 bp, synthetic construct
  source 1..21: mol_type = other DNA; note = shDDX54
ccggtttatcagcagctctta